European Patent Application EP 4 442 276 A1, published October 9, 2024. Title: COMBINED ANTIBODIES AGAINST SARBECOVIRUSES AND USES THEREOF. Applicant: INSTITUT PASTEUR. The sequence listing filed with the application follows.

SEQUENCE LISTING (66 sequences)

SEQ ID NO: 1 - protein, 5 aa, synthetic construct
  REGION 1..5: note = >CDRH1
DYYMS

SEQ ID NO: 2 - protein, 17 aa, synthetic construct
  REGION 1..17: note = >CDRH2
YISSSGSVQYYADSVKG

SEQ ID NO: 3 - protein, 14 aa, synthetic construct
  REGION 1..14: note = >CDRH3
YYYDSSGYWKRLDY

SEQ ID NO: 4 - protein, 11 aa, synthetic construct
  REGION 1..11: note = >CDRL1
RASQSISRYLN

SEQ ID NO: 5 - protein, 7 aa, synthetic construct
  REGION 1..7: note = >CDRL2
AASSLQS

SEQ ID NO: 6 - protein, 9 aa, synthetic construct
  REGION 1..9: note = >CDRL3
QQSYSTPLT

SEQ ID NO: 7 - protein, 30 aa, synthetic construct
  REGION 1..30: note = >HFW1
EVQLVESGGGLVKPGGSLRLSCAASGFTFS

SEQ ID NO: 8 - protein, 14 aa, synthetic construct
  REGION 1..14: note = >HFW2
WIRQAPGKGLEWVS

SEQ ID NO: 9 - protein, 32 aa, synthetic construct
  REGION 1..32: note = >HFW3
RFTISRDNAKNSLYLQMNSLRAEDTAVYYCAR

SEQ ID NO: 10 - protein, 11 aa, synthetic construct
  REGION 1..11: note = >HFW4
WGQGTLVTVSS

SEQ ID NO: 11 - protein, 23 aa, synthetic construct
  REGION 1..23: note = >LFW1
DIQMTQSPSSLSASVGDRVTITC

SEQ ID NO: 12 - protein, 15 aa, synthetic construct
  REGION 1..15: note = >LFW2
WYQQKPGKAPKLLIY

SEQ ID NO: 13 - protein, 32 aa, synthetic construct
  REGION 1..32: note = >LFW3
GVPSRFSGSGSGTDFTLTISSLQPEDFATYHC

SEQ ID NO: 14 - protein, 10 aa, synthetic construct
  REGION 1..10: note = >LFW4
FGGGTKVEIK

SEQ ID NO: 15 - protein, 123 aa, synthetic construct
  REGION 1..123: note = >VH
EVQLVESGGGLVKPGGSLRLSCAASGFTFSDYYMSWIRQAPGKGLEWVSYISSSGSVQYYADSVKGRFTISRDNAKNSLYLQMNSLRAEDTAVYYCARYYYDSSGYWKRLDYWGQGTLVTVSS

SEQ ID NO: 16 - protein, 107 aa, synthetic construct
  REGION 1..107: note = >VL
DIQMTQSPSSLSASVGDRVTITCRASQSISRYLNWYQQKPGKAPKLLIYAASSLQSGVPSRFSGSGSGTDFTLTISSLQPEDFATYHCQQSYSTPLTFGGGTKVEIK

SEQ ID NO: 17 - protein, 214 aa, synthetic construct
  REGION 1..214: note = >FL-Light Chain
DIQMTQSPSSLSASVGDRVTITCRASQSISRYLNWYQQKPGKAPKLLIYAASSLQSGVPSRFSGSGSGTDFTLTISSLQPEDFATYHCQQSYSTPLTFGGGTKVEIKRTVAAPSVFIFPPSDEQLKSGTASVVCLLNNFYPREAKVQWKVDNALQSGNSQESVTEQDSKDSTYSLSSTLTLSKADYEKHKVYACEVTHQGLSSPVTKSFNRGEC

SEQ ID NO: 18 - protein, 453 aa, synthetic construct
  REGION 1..453: note = >FL-heavy Chain
EVQLVESGGGLVKPGGSLRLSCAASGFTFSDYYMSWIRQAPGKGLEWVSYISSSGSVQYYADSVKGRFTISRDNAKNSLYLQMNSLRAEDTAVYYCARYYYDSSGYWKRLDYWGQGTLVTVSSASTKGPSVFPLAPSSKSTSGGTAALGCLVKDYFPEPVTVSWNSGALTSGVHTFPAVLQSSGLYSLSSVVTVPSSSLGTQTYICNVNHKPSNTKVDKRVEPKSCDKTHTCPPCPAPELLGGPSVFLFPPKPKDTLMISRTPEVTCVVVDVSHEDPEVKFNWYVDGVEVHNAKTKPREEQYNSTYRVVSVLTVLHQDWLNGKEYKCKVSNKALPAPIEKTISKAKGQPREPQVYTLPPSREEMTKNQVSLTCLVKGFYPSDIAVEWESNGQPENNYKTTPPVLDSDGSFFLYSKLTVDKSRWQQGNVFSCSVMHEALHNHYTQKSLSLSPGK

SEQ ID NO: 19 - DNA, 321 bp, synthetic construct
  misc_feature 1..321: note = >VLnucleotide
  source 1..321: mol_type = other DNA
gacatccagatgacccagtctccatcctccctgtctgcatctgtaggagacagagtcaccatcacttgccgggcaagtcagagcattagcaggtatttaaattggtatcagcagaaaccagggaaagcccctaagctcctgatctatgctgcatccagtttgcaaagtggggtcccatcaaggttcagtggcagtggatctgggacagatttcacgctcaccatcagcagtctgcaacctgaagattttgcaacttaccactgtcaacagagttacagtaccccgctcactttcggcggagggaccaaggtggagatcaaa

SEQ ID NO: 20 - DNA, 369 bp, synthetic construct
  misc_feature 1..369: note = >VHnucleotide
  source 1..369: mol_type = other DNA
gaggtgcagctggtggagtctgggggaggcttggtcaagcctggagggtccctgagactctcctgtgcagcctctggattcaccttcagtgactactacatgagctggatccgccaggctccagggaaggggctggagtgggtttcatacattagtagtagtggtagtgtccaatactacgcagactctgtgaagggccgattcaccatctccagggacaacgccaagaactctctgtatctgcaaatgaacagcctgagagccgaggacacggccgtgtattactgtgcgaggtattactatgatagtagtggttattggaaaaggttggactactggggccagggaaccctggtcaccgtctcctca

SEQ ID NO: 21 - protein, 20 aa, synthetic construct
  REGION 1..20: note = >HR2peptide1
DVDLGDISGINASVVNIQKE

SEQ ID NO: 22 - protein, 20 aa, synthetic construct
  REGION 1..20: note = >HR2peptide2
DISGINASVVNIQKEIDRLN

SEQ ID NO: 23 - protein, 20 aa, synthetic construct
  REGION 1..20: note = >HR2peptide3
NASVVNIQKEIDRLNEVAKN

SEQ ID NO: 24 - protein, 20 aa, synthetic construct
  REGION 1..20: note = >HR2peptide4
NIQKEIDRLNEVAKNLNESL

SEQ ID NO: 25 - protein, 20 aa, synthetic construct
  REGION 1..20: note = >HR2peptide5
IDRLNEVAKNLNESLIDLQE

SEQ ID NO: 26 - protein, 20 aa, synthetic construct
  REGION 1..20: note = >HR2peptide6
EVAKNLNESLIDLQELGKYE

SEQ ID NO: 27 - protein, 20 aa, synthetic construct
  REGION 1..20: note = >HR2peptide7
LNESLIDLQELGKYEQYIKW

SEQ ID NO: 28 - protein, 16 aa, synthetic construct
  REGION 1..16: note = >HR2peptide8
IDLQELGKYEQYIKWP

SEQ ID NO: 29 - protein, 5 aa, synthetic construct
  REGION 1..5: note = >29
TSAVQ

SEQ ID NO: 30 - protein, 17 aa, synthetic construct
  REGION 1..17: note = >30
WIVVGSGNTNYAQKFQE

SEQ ID NO: 31 - protein, 14 aa, synthetic construct
  REGION 1..14: note = >31
PYCSGGTCLDGFDI

SEQ ID NO: 32 - protein, 12 aa, synthetic construct
  REGION 1..12: note = >32
RASQSVSRSYLA

SEQ ID NO: 33 - protein, 7 aa, synthetic construct
  REGION 1..7: note = >33
SASSRAT

SEQ ID NO: 34 - protein, 9 aa, synthetic construct
  REGION 1..9: note = >34
QQYGSSPWT

SEQ ID NO: 35 - protein, 5 aa, synthetic construct
  REGION 1..5: note = >35
SNYMN

SEQ ID NO: 36 - protein, 16 aa, synthetic construct
  REGION 1..16: note = >36
VIYSGGSTFYADSVKG

SEQ ID NO: 37 - protein, 9 aa, synthetic construct
  REGION 1..9: note = >37
DLGPMGFDI

SEQ ID NO: 38 - protein, 11 aa, synthetic construct
  REGION 1..11: note = >38
RASQGISSYLA

SEQ ID NO: 39 - protein, 7 aa, synthetic construct
  REGION 1..7: note = >39
AASTLQS

SEQ ID NO: 40 - protein, 10 aa, synthetic construct
  REGION 1..10: note = >40
QQLNSDPPVT

SEQ ID NO: 41 - protein, 5 aa, synthetic construct
  REGION 1..5: note = >41
SNYMS

SEQ ID NO: 42 - protein, 16 aa, synthetic construct
  REGION 1..16: note = >42
VIYPGGSTFYADSVKG

SEQ ID NO: 43 - protein, 9 aa, synthetic construct
  REGION 1..9: note = >43
DLVVYGMDV

SEQ ID NO: 44 - protein, 12 aa, synthetic construct
  REGION 1..12: note = >44
RASQSVSSSYLA

SEQ ID NO: 45 - protein, 7 aa, synthetic construct
  REGION 1..7: note = >45
GASSRAT

SEQ ID NO: 46 - protein, 5 aa, synthetic construct
  REGION 1..5: note = >46
QQGVT

SEQ ID NO: 47 - protein, 5 aa, synthetic construct
  REGION 1..5: note = >47
RNYMS

SEQ ID NO: 48 - protein, 16 aa, synthetic construct
  REGION 1..16: note = >48
VIYSGGSTFYADSVKG

SEQ ID NO: 49 - protein, 9 aa, synthetic construct
  REGION 1..9: note = >49
DGDYYGMDV

SEQ ID NO: 50 - protein, 11 aa, synthetic construct
  REGION 1..11: note = >50
RASQGISSFLA

SEQ ID NO: 51 - protein, 7 aa, synthetic construct
  REGION 1..7: note = >51
GASTLQS

SEQ ID NO: 52 - protein, 10 aa, synthetic construct
  REGION 1..10: note = >52
QRLDSYPPIT

SEQ ID NO: 53 - protein, 5 aa, synthetic construct
  REGION 1..5: note = >53
SNYMS

SEQ ID NO: 54 - protein, 16 aa, synthetic construct
  REGION 1..16: note = >54
LIYSGGSTYYADSVKG

SEQ ID NO: 55 - protein, 9 aa, synthetic construct
  REGION 1..9: note = >55
DLNYYGMDV

SEQ ID NO: 56 - protein, 11 aa, synthetic construct
  REGION 1..11: note = >56
RASQGISSYLA

SEQ ID NO: 57 - protein, 7 aa, synthetic construct
  REGION 1..7: note = >57
AASTLQS

SEQ ID NO: 58 - protein, 10 aa, synthetic construct
  REGION 1..10: note = >58
QQLDSYSPFT

SEQ ID NO: 59 - protein, 5 aa, synthetic construct
  REGION 1..5: note = >59
SSAVQ

SEQ ID NO: 60 - protein, 17 aa, synthetic construct
  REGION 1..17: note = >60
WIVVGSGNTNYAQKFQE

SEQ ID NO: 61 - protein, 14 aa, synthetic construct
  REGION 1..14: note = >61
PHCSSTSCYDAFDI

SEQ ID NO: 62 - protein, 12 aa, synthetic construct
  REGION 1..12: note = >62
RASQSVSSSYLA

SEQ ID NO: 63 - protein, 7 aa, synthetic construct
  REGION 1..7: note = >63
GASSRAT

SEQ ID NO: 64 - protein, 9 aa, synthetic construct
  REGION 1..9: note = >64
QQYGRSPWT

SEQ ID NO: 65 - protein, 51 aa, synthetic construct
  REGION 1..51: note = >HR2region
DVDLGDISGINASVVNIQKEIDRLNEVAKNLNESLIDLQELGKYEQYIKWP

SEQ ID NO: 66 - protein, 22 aa, synthetic construct
  REGION 1..22: note = >FP
KRSFIEDLLFNKVTLADAGFIK